European Patent Application EP 4 393 940 A1, published July 3, 2024. Title: GDF15 FUSION PROTEINS AND USES THEREOF. Applicant: Sunshine Lake Pharma Co., Ltd. Application WO. The sequence listing filed with the application follows.

SEQUENCE LISTING (127 sequences)

SEQ ID NO: 1 - protein, 210 aa, synthetic construct
GPSVFLFPPKPKDTLMISRTPEVTCVVVDVSQEDPEVQFNWYVDGVEVHNAKTKPREEQFNSTYRVVSVLTVLHQDWLNGKEYKCKVSNKGLPSSIEKTISKAKGQPREPQVYTLPPSQEEMTKNQVSLTCLVKGFYPSDIAVEWESNGQPENNYKTTPPVLDSDGSFFLYSRLTVDKSRWQEGNVFSCSVMHEALHNHYTQESLSLSLG

SEQ ID NO: 2 - protein, 211 aa, synthetic construct
GGPSVFLFPPKPKDTLMISRTPEVTCVVVDVSQEDPEVQFNWYVDGVEVHNAKTKPREEQFNSTYRVVSVLTVLHQDWLNGKEYKCKVSNKGLPSSIEKTISKAKGQPREPQVYTLPPSQEEMTKNQVSLTCLVKGFYPSDIAVEWESNGQPENNYKTTPPVLDSDGSFFLYSRLTVDKSRWQEGNVFSCSVMHEALHNHYTQESLSLSLG

SEQ ID NO: 3 - protein, 214 aa, synthetic construct
EAAGGPSVFLFPPKPKDTLMISRTPEVTCVVVDVSQEDPEVQFNWYVDGVEVHNAKTKPREEQFNSTYRVVSVLTVLHQDWLNGKEYKCKVSNKGLPSSIEKTISKAKGQPREPQVYTLPPSQEEMTKNQVSLTCLVKGFYPSDIAVEWESNGQPENNYKTTPPVLDSDGSFFLYSRLTVDKSRWQEGNVFSCSVMHEALHNHYTQESLSLSLG

SEQ ID NO: 4 - protein, 216 aa, synthetic construct
APEAAGGPSVFLFPPKPKDTLMISRTPEVTCVVVDVSQEDPEVQFNWYVDGVEVHNAKTKPREEQFNSTYRVVSVLTVLHQDWLNGKEYKCKVSNKGLPSSIEKTISKAKGQPREPQVYTLPPSQEEMTKNQVSLTCLVKGFYPSDIAVEWESNGQPENNYKTTPPVLDSDGSFFLYSRLTVDKSRWQEGNVFSCSVMHEALHNHYTQESLSLSLG

SEQ ID NO: 5 - protein, 210 aa, synthetic construct
GPSVFLFPPKPKDTLMISRTPEVTCVVVDVSQEDPEVQFNWYVDGVEVHNAKTKPREEQFNSTYRVVSVLTVLHQDWLNGKEYKCKVSNKGLPSSIEKTISKAKGQPREPQVYTLPPSQEEMTKNQVSLTCLVKGFYPSDIAVEWESNGQPENNYKTTPPVLDSDGSFFLYSRLTVDKSRWQEGNVFSCSVMHEALHNHYTQDSLSLSLG

SEQ ID NO: 6 - protein, 211 aa, synthetic construct
GGPSVFLFPPKPKDTLMISRTPEVTCVVVDVSQEDPEVQFNWYVDGVEVHNAKTKPREEQFNSTYRVVSVLTVLHQDWLNGKEYKCKVSNKGLPSSIEKTISKAKGQPREPQVYTLPPSQEEMTKNQVSLTCLVKGFYPSDIAVEWESNGQPENNYKTTPPVLDSDGSFFLYSRLTVDKSRWQEGNVFSCSVMHEALHNHYTQDSLSLSLG

SEQ ID NO: 7 - protein, 214 aa, synthetic construct
EAAGGPSVFLFPPKPKDTLMISRTPEVTCVVVDVSQEDPEVQFNWYVDGVEVHNAKTKPREEQFNSTYRVVSVLTVLHQDWLNGKEYKCKVSNKGLPSSIEKTISKAKGQPREPQVYTLPPSQEEMTKNQVSLTCLVKGFYPSDIAVEWESNGQPENNYKTTPPVLDSDGSFFLYSRLTVDKSRWQEGNVFSCSVMHEALHNHYTQDSLSLSLG

SEQ ID NO: 8 - protein, 216 aa, synthetic construct
APEAAGGPSVFLFPPKPKDTLMISRTPEVTCVVVDVSQEDPEVQFNWYVDGVEVHNAKTKPREEQFNSTYRVVSVLTVLHQDWLNGKEYKCKVSNKGLPSSIEKTISKAKGQPREPQVYTLPPSQEEMTKNQVSLTCLVKGFYPSDIAVEWESNGQPENNYKTTPPVLDSDGSFFLYSRLTVDKSRWQEGNVFSCSVMHEALHNHYTQDSLSLSLG

SEQ ID NO: 9 - protein, 210 aa, synthetic construct
GPSVFLFPPKPKDTLMISRTPEVTCVVVDVSQEDPEVQFNWYVDGVEVHNAKTKPREEQFNSTYRVVSVLTVLHQDWLNGKEYKCKVSNKGLPSSIEKTISKAKGQPREPQVYTLPPSQKEMTKNQVSLTCLVKGFYPSDIAVEWESNGQPENNYKTTPPVLDSDGSFFLYSRLTVDKSRWQEGNVFSCSVMHEALHNHYTQKSLSLSLG

SEQ ID NO: 10 - protein, 211 aa, synthetic construct
GGPSVFLFPPKPKDTLMISRTPEVTCVVVDVSQEDPEVQFNWYVDGVEVHNAKTKPREEQFNSTYRVVSVLTVLHQDWLNGKEYKCKVSNKGLPSSIEKTISKAKGQPREPQVYTLPPSQKEMTKNQVSLTCLVKGFYPSDIAVEWESNGQPENNYKTTPPVLDSDGSFFLYSRLTVDKSRWQEGNVFSCSVMHEALHNHYTQKSLSLSLG

SEQ ID NO: 11 - protein, 214 aa, synthetic construct
EAAGGPSVFLFPPKPKDTLMISRTPEVTCVVVDVSQEDPEVQFNWYVDGVEVHNAKTKPREEQFNSTYRVVSVLTVLHQDWLNGKEYKCKVSNKGLPSSIEKTISKAKGQPREPQVYTLPPSQKEMTKNQVSLTCLVKGFYPSDIAVEWESNGQPENNYKTTPPVLDSDGSFFLYSRLTVDKSRWQEGNVFSCSVMHEALHNHYTQKSLSLSLG

SEQ ID NO: 12 - protein, 216 aa, synthetic construct
APEAAGGPSVFLFPPKPKDTLMISRTPEVTCVVVDVSQEDPEVQFNWYVDGVEVHNAKTKPREEQFNSTYRVVSVLTVLHQDWLNGKEYKCKVSNKGLPSSIEKTISKAKGQPREPQVYTLPPSQKEMTKNQVSLTCLVKGFYPSDIAVEWESNGQPENNYKTTPPVLDSDGSFFLYSRLTVDKSRWQEGNVFSCSVMHEALHNHYTQKSLSLSLG

SEQ ID NO: 13 - protein, 210 aa, synthetic construct
GPSVFLFPPKPKDTLMISRTPEVTCVVVDVSQEDPEVQFNWYVDGVEVHNAKTKPREEQFNSTYRVVSVLTVLHQDWLNGKEYKCKVSNKGLPSSIEKTISKAKGQPREPQVYTLPPSQREMTKNQVSLTCLVKGFYPSDIAVEWESNGQPENNYKTTPPVLDSDGSFFLYSRLTVDKSRWQEGNVFSCSVMHEALHNHYTQKSLSLSLG

SEQ ID NO: 14 - protein, 211 aa, synthetic construct
GGPSVFLFPPKPKDTLMISRTPEVTCVVVDVSQEDPEVQFNWYVDGVEVHNAKTKPREEQFNSTYRVVSVLTVLHQDWLNGKEYKCKVSNKGLPSSIEKTISKAKGQPREPQVYTLPPSQREMTKNQVSLTCLVKGFYPSDIAVEWESNGQPENNYKTTPPVLDSDGSFFLYSRLTVDKSRWQEGNVFSCSVMHEALHNHYTQKSLSLSLG

SEQ ID NO: 15 - protein, 214 aa, synthetic construct
EAAGGPSVFLFPPKPKDTLMISRTPEVTCVVVDVSQEDPEVQFNWYVDGVEVHNAKTKPREEQFNSTYRVVSVLTVLHQDWLNGKEYKCKVSNKGLPSSIEKTISKAKGQPREPQVYTLPPSQREMTKNQVSLTCLVKGFYPSDIAVEWESNGQPENNYKTTPPVLDSDGSFFLYSRLTVDKSRWQEGNVFSCSVMHEALHNHYTQKSLSLSLG

SEQ ID NO: 16 - protein, 216 aa, synthetic construct
APEAAGGPSVFLFPPKPKDTLMISRTPEVTCVVVDVSQEDPEVQFNWYVDGVEVHNAKTKPREEQFNSTYRVVSVLTVLHQDWLNGKEYKCKVSNKGLPSSIEKTISKAKGQPREPQVYTLPPSQREMTKNQVSLTCLVKGFYPSDIAVEWESNGQPENNYKTTPPVLDSDGSFFLYSRLTVDKSRWQEGNVFSCSVMHEALHNHYTQKSLSLSLG

SEQ ID NO: 17 - protein, 216 aa, synthetic construct
APEAAGGPSVFLFPPKPKDTLMISRTPEVTCVVVDVSQEDPEVQFNWYVDGVEVHNAKTKPREEQFNSTYRVVSVLTVLHQDWLNGKEYKCKVSNKGLPSSIEKTISKAKGQPREPQVYTLPPSQEEMTKNQVSLTCLVKGFYPSDIAVEWESNGQPENNYKTTPPVLDSDGSFFLYSRLTVDKSRWQEGNVFSCSVMHEALHNHYTQQSLSLSLG

SEQ ID NO: 18 - protein, 216 aa, synthetic construct
APEAAGGPSVFLFPPKPKDTLMISRTPEVTCVVVDVSQEDPEVQFNWYVDGVEVHNAKTKPREEQFNSTYRVVSVLTVLHQDWLNGKEYKCKVSNKGLPSSIEKTISKAKGQPREPQVYTLPPSQEEMTKNQVSLTCLVKGFYPSDIAVEWESNGQPENNYKTTPPVLDSDGSFFLYSRLTVDKSRWQEGNVFSCSVMHEALHNHYTQNSLSLSLG

SEQ ID NO: 19 - protein, 216 aa, synthetic construct
APEAAGGPSVFLFPPKPKDTLMISRTPEVTCVVVDVSQEDPEVQFNWYVDGVEVHNAKTKPREEQFNSTYRVVSVLTVLHQDWLNGKEYKCKVSNKGLPSSIEKTISKAKGQPREPQVYTLPPSQEEMTKNQVSLTCLVKGFYPSDIAVEWESNGQPENNYKTTPPVLDSDGSFFLYSRLTVDKSRWQEGNVFSCSVMHEALHNHYTQASLSLSLG

SEQ ID NO: 20 - protein, 216 aa, synthetic construct
APEAAGGPSVFLFPPKPKDTLMISRTPEVTCVVVDVSQEDPEVQFNWYVDGVEVHNAKTKPREEQFNSTYRVVSVLTVLHQDWLNGKEYKCKVSNKGLPSSIEKTISKAKGQPREPQVYTLPPSQQEMTKNQVSLTCLVKGFYPSDIAVEWESNGQPENNYKTTPPVLDSDGSFFLYSRLTVDKSRWQEGNVFSCSVMHEALHNHYTQKSLSLSLG

SEQ ID NO: 21 - protein, 216 aa, synthetic construct
APEAAGGPSVFLFPPKPKDTLMISRTPEVTCVVVDVSQEDPEVQFNWYVDGVEVHNAKTKPREEQFNSTYRVVSVLTVLHQDWLNGKEYKCKVSNKGLPSSIEKTISKAKGQPREPQVYTLPPSQNEMTKNQVSLTCLVKGFYPSDIAVEWESNGQPENNYKTTPPVLDSDGSFFLYSRLTVDKSRWQEGNVFSCSVMHEALHNHYTQKSLSLSLG

SEQ ID NO: 22 - protein, 216 aa, synthetic construct
APEAAGGPSVFLFPPKPKDTLMISRTPEVTCVVVDVSQEDPEVQFNWYVDGVEVHNAKTKPREEQFNSTYRVVSVLTVLHQDWLNGKEYKCKVSNKGLPSSIEKTISKAKGQPREPQVYTLPPSQAEMTKNQVSLTCLVKGFYPSDIAVEWESNGQPENNYKTTPPVLDSDGSFFLYSRLTVDKSRWQEGNVFSCSVMHEALHNHYTQKSLSLSLG

SEQ ID NO: 23 - protein, 214 aa, synthetic construct
EAAGGPSVFLFPPKPKDTLMISRTPEVTCVVVDVSQEDPEVQFNWYVDGVEVHNAKTKPREEQFNSTYRVVSVLTVLHQDWLNGKEYKCKVSNKGLPSSIEKTISKAKGQPREPQVYTLPPSQEEMTKNQVSLTCLVKGFYPSDIAVEWESNGQPENNYKTTPPVLDSDGSFFLYSRLTVDKSRWQEGNVFSCSVMHEALHNHYTQKSLSLSLG

SEQ ID NO: 24 - protein, 214 aa, synthetic construct
EAAGGPSVFLFPPKPKDTLMISRTPEVTCVVVDVSQEDPEVQFNWYVDGVEVHNAKTKPREEQFNSTYRVVSVLTVLHQDWLNGKEYKCKVSNKGLPSSIEKTISKAKGQPREPQVYTLPPSQEEMTKNQVSLTCLVKGFYPSDIAVEWESNGQPENNYKTTPPVLDSDGSFQLESRLTVDKSRWQEGNVFSCSVMHEALHNHYTQKSLSLSLG

SEQ ID NO: 25 - protein, 216 aa, synthetic construct
APEAAGGPSVFLFPPKPKDTLMISRTPEVTCVVVDVSQEDPEVQFNWYVDGVEVHNAKTKPREEQFNSTYRVVSVLTVLHQDWLNGKEYKCKVSNKGLPSSIEKTISKAKGQPREPQVYTLPPSQEEMTKNQVSLTCLVKGFYPSDIAVEWESNGQPENNYKTTPPVLDSDGSFFLYSRLTVDKSRWQEGNVFSCSVMHEALHNHYTQKSLSLSLG

SEQ ID NO: 26 - protein, 211 aa, synthetic construct
GGPSVFLFPPKPKDTLMISRTPEVTCVVVDVSQEDPEVQFNWYVDGVEVHNAKTKPREEQFNSTYRVVSVLTVLHQDWLNGKEYKCKVSNKGLPSSIEKTISKAKGQPREPQVYTLPPSQEEMTKNQVSLTCLVKGFYPSDIAVEWESNGQPENNYKTTPPVLDSDGSFFLYSRLTVDKSRWQEGNVFSCSVMHEALHNHYTQKSLSLSLG

SEQ ID NO: 27 - protein, 229 aa, synthetic construct
AESKYGPPCPPCPAPEAAGGPSVFLFPPKPKDTLMISRTPEVTCVVVDVSQEDPEVQFNWYVDGVEVHNAKTKPREEQFNSTYRVVSVLTVLHQDWLNGKEYKCKVSNKGLPSSIEKTISKAKGQPREPQVYTLPPSQEEMTKNQVSLTCLVKGFYPSDIAVEWESNGQPENNYKTTPPVLDSDGSFFLYSRLTVDKSRWQEGNVFSCSVMHEALHNHYTQESLSLSLG

SEQ ID NO: 28 - protein, 211 aa, synthetic construct
GGPSVFLFPPKPKDTLMISRTPEVTCVVVDVSQEDPEVQFNWYVDGVEVHNAKTKPREEQFNSTYRVVSVLTVLHQDWLNGKEYKCKVSNKGLPSSIEKTISKAKGQPREPQVYTLPPSQEEMTKNQVSLTCLVKGFYPSDIAVEWESNGQPENNYKTTPPVLDSDGSFQLESRLTVDKSRWQEGNVFSCSVMHEALHNHYTQESLSLSLG

SEQ ID NO: 29 - protein, 210 aa, synthetic construct
GPSVFLFPPKPKDTLMISRTPEVTCVVVDVSHEDPEVKFNWYVDGVEVHNAKTKPREEQYNSTYRVVSVLTVLHQDWLNGKEYKCKVSNKALPAPIEKTISKAKGQPREPQVYTLPPSREEMTKNQVSLTCLVKGFYPSDIAVEWESNGQPENNYKTTPPVLDSDGSFFLYSKLTVDKSRWQQGNVFSCSVMHEALHNHYTQESLSLSPG

SEQ ID NO: 30 - protein, 211 aa, synthetic construct
GGPSVFLFPPKPKDTLMISRTPEVTCVVVDVSHEDPEVKFNWYVDGVEVHNAKTKPREEQYNSTYRVVSVLTVLHQDWLNGKEYKCKVSNKALPAPIEKTISKAKGQPREPQVYTLPPSREEMTKNQVSLTCLVKGFYPSDIAVEWESNGQPENNYKTTPPVLDSDGSFFLYSKLTVDKSRWQQGNVFSCSVMHEALHNHYTQESLSLSPG

SEQ ID NO: 31 - protein, 214 aa, synthetic construct
EAAGGPSVFLFPPKPKDTLMISRTPEVTCVVVDVSHEDPEVKFNWYVDGVEVHNAKTKPREEQYNSTYRVVSVLTVLHQDWLNGKEYKCKVSNKALPAPIEKTISKAKGQPREPQVYTLPPSREEMTKNQVSLTCLVKGFYPSDIAVEWESNGQPENNYKTTPPVLDSDGSFFLYSKLTVDKSRWQQGNVFSCSVMHEALHNHYTQESLSLSPG

SEQ ID NO: 32 - protein, 216 aa, synthetic construct
APEAAGGPSVFLFPPKPKDTLMISRTPEVTCVVVDVSHEDPEVKFNWYVDGVEVHNAKTKPREEQYNSTYRVVSVLTVLHQDWLNGKEYKCKVSNKALPAPIEKTISKAKGQPREPQVYTLPPSREEMTKNQVSLTCLVKGFYPSDIAVEWESNGQPENNYKTTPPVLDSDGSFFLYSKLTVDKSRWQQGNVFSCSVMHEALHNHYTQESLSLSPG

SEQ ID NO: 33 - protein, 210 aa, synthetic construct
GPSVFLFPPKPKDTLMISRTPEVTCVVVDVSHEDPEVKFNWYVDGVEVHNAKTKPREEQYNSTYRVVSVLTVLHQDWLNGKEYKCKVSNKALPAPIEKTISKAKGQPREPQVYTLPPSREEMTKNQVSLTCLVKGFYPSDIAVEWESNGQPENNYKTTPPVLDSDGSFFLYSKLTVDKSRWQQGNVFSCSVMHEALHNHYTQDSLSLSPG

SEQ ID NO: 34 - protein, 211 aa, synthetic construct
GGPSVFLFPPKPKDTLMISRTPEVTCVVVDVSHEDPEVKFNWYVDGVEVHNAKTKPREEQYNSTYRVVSVLTVLHQDWLNGKEYKCKVSNKALPAPIEKTISKAKGQPREPQVYTLPPSREEMTKNQVSLTCLVKGFYPSDIAVEWESNGQPENNYKTTPPVLDSDGSFFLYSKLTVDKSRWQQGNVFSCSVMHEALHNHYTQDSLSLSPG

SEQ ID NO: 35 - protein, 214 aa, synthetic construct
EAAGGPSVFLFPPKPKDTLMISRTPEVTCVVVDVSHEDPEVKFNWYVDGVEVHNAKTKPREEQYNSTYRVVSVLTVLHQDWLNGKEYKCKVSNKALPAPIEKTISKAKGQPREPQVYTLPPSREEMTKNQVSLTCLVKGFYPSDIAVEWESNGQPENNYKTTPPVLDSDGSFFLYSKLTVDKSRWQQGNVFSCSVMHEALHNHYTQDSLSLSPG

SEQ ID NO: 36 - protein, 216 aa, synthetic construct
APEAAGGPSVFLFPPKPKDTLMISRTPEVTCVVVDVSHEDPEVKFNWYVDGVEVHNAKTKPREEQYNSTYRVVSVLTVLHQDWLNGKEYKCKVSNKALPAPIEKTISKAKGQPREPQVYTLPPSREEMTKNQVSLTCLVKGFYPSDIAVEWESNGQPENNYKTTPPVLDSDGSFFLYSKLTVDKSRWQQGNVFSCSVMHEALHNHYTQDSLSLSPG

SEQ ID NO: 37 - protein, 210 aa, synthetic construct
GPSVFLFPPKPKDTLMISRTPEVTCVVVDVSHEDPEVKFNWYVDGVEVHNAKTKPREEQYNSTYRVVSVLTVLHQDWLNGKEYKCKVSNKALPAPIEKTISKAKGQPREPQVYTLPPSRKEMTKNQVSLTCLVKGFYPSDIAVEWESNGQPENNYKTTPPVLDSDGSFFLYSKLTVDKSRWQQGNVFSCSVMHEALHNHYTQKSLSLSPG

SEQ ID NO: 38 - protein, 211 aa, synthetic construct
GGPSVFLFPPKPKDTLMISRTPEVTCVVVDVSHEDPEVKFNWYVDGVEVHNAKTKPREEQYNSTYRVVSVLTVLHQDWLNGKEYKCKVSNKALPAPIEKTISKAKGQPREPQVYTLPPSRKEMTKNQVSLTCLVKGFYPSDIAVEWESNGQPENNYKTTPPVLDSDGSFFLYSKLTVDKSRWQQGNVFSCSVMHEALHNHYTQKSLSLSPG

SEQ ID NO: 39 - protein, 214 aa, synthetic construct
EAAGGPSVFLFPPKPKDTLMISRTPEVTCVVVDVSHEDPEVKFNWYVDGVEVHNAKTKPREEQYNSTYRVVSVLTVLHQDWLNGKEYKCKVSNKALPAPIEKTISKAKGQPREPQVYTLPPSRKEMTKNQVSLTCLVKGFYPSDIAVEWESNGQPENNYKTTPPVLDSDGSFFLYSKLTVDKSRWQQGNVFSCSVMHEALHNHYTQKSLSLSPG

SEQ ID NO: 40 - protein, 216 aa, synthetic construct
APEAAGGPSVFLFPPKPKDTLMISRTPEVTCVVVDVSHEDPEVKFNWYVDGVEVHNAKTKPREEQYNSTYRVVSVLTVLHQDWLNGKEYKCKVSNKALPAPIEKTISKAKGQPREPQVYTLPPSRKEMTKNQVSLTCLVKGFYPSDIAVEWESNGQPENNYKTTPPVLDSDGSFFLYSKLTVDKSRWQQGNVFSCSVMHEALHNHYTQKSLSLSPG

SEQ ID NO: 41 - protein, 210 aa, synthetic construct
GPSVFLFPPKPKDTLMISRTPEVTCVVVDVSHEDPEVKFNWYVDGVEVHNAKTKPREEQYNSTYRVVSVLTVLHQDWLNGKEYKCKVSNKALPAPIEKTISKAKGQPREPQVYTLPPSRREMTKNQVSLTCLVKGFYPSDIAVEWESNGQPENNYKTTPPVLDSDGSFFLYSKLTVDKSRWQQGNVFSCSVMHEALHNHYTQKSLSLSPG

SEQ ID NO: 42 - protein, 211 aa, synthetic construct
GGPSVFLFPPKPKDTLMISRTPEVTCVVVDVSHEDPEVKFNWYVDGVEVHNAKTKPREEQYNSTYRVVSVLTVLHQDWLNGKEYKCKVSNKALPAPIEKTISKAKGQPREPQVYTLPPSRREMTKNQVSLTCLVKGFYPSDIAVEWESNGQPENNYKTTPPVLDSDGSFFLYSKLTVDKSRWQQGNVFSCSVMHEALHNHYTQKSLSLSPG

SEQ ID NO: 43 - protein, 214 aa, synthetic construct
EAAGGPSVFLFPPKPKDTLMISRTPEVTCVVVDVSHEDPEVKFNWYVDGVEVHNAKTKPREEQYNSTYRVVSVLTVLHQDWLNGKEYKCKVSNKALPAPIEKTISKAKGQPREPQVYTLPPSRREMTKNQVSLTCLVKGFYPSDIAVEWESNGQPENNYKTTPPVLDSDGSFFLYSKLTVDKSRWQQGNVFSCSVMHEALHNHYTQKSLSLSPG

SEQ ID NO: 44 - protein, 216 aa, synthetic construct
APEAAGGPSVFLFPPKPKDTLMISRTPEVTCVVVDVSHEDPEVKFNWYVDGVEVHNAKTKPREEQYNSTYRVVSVLTVLHQDWLNGKEYKCKVSNKALPAPIEKTISKAKGQPREPQVYTLPPSRREMTKNQVSLTCLVKGFYPSDIAVEWESNGQPENNYKTTPPVLDSDGSFFLYSKLTVDKSRWQQGNVFSCSVMHEALHNHYTQKSLSLSPG

SEQ ID NO: 45 - protein, 216 aa, synthetic construct
APEAAGGPSVFLFPPKPKDTLMISRTPEVTCVVVDVSQEDPEVQFNWYVDGVEVHNAKTKPREEQFNSTYRVVSVLTVLHQDWLNGKEYKCKVSNKGLPSSIEKTISKAKGQPREPQVYTLPPSQQEMTKNQVSLTCLVKGFYPSDIAVEWESNGQPENNYKTTPPVLDSDGSFFLYSRLTVDKSRWQEGNVFSCSVMHEALHNHYTQQSLSLSLG

SEQ ID NO: 46 - protein, 112 aa, synthetic construct
ARNGDHCPLGPGRCCRLHTVRASLEDLGWADWVLSPREVQVTMCIGACPSQFRAANMHAQIKTSLHRLKPDTVPAPCCVPASYNPMVLIQKTDTGVSLQTYDDLLAKDCHCI

SEQ ID NO: 47 - protein, 109 aa, synthetic construct
GDHCPLGPGRCCRLHTVRASLEDLGWADWVLSPREVQVTMCIGACPSQFRAANMHAQIKTSLHRLKPDTVPAPCCVPASYNPMVLIQKTDTGVSLQTYDDLLAKDCHCI

SEQ ID NO: 48 - protein, 108 aa, synthetic construct
DHCPLGPGRCCRLHTVRASLEDLGWADWVLSPREVQVTMCIGACPSQFRAANMHAQIKTSLHRLKPDTVPAPCCVPASYNPMVLIQKTDTGVSLQTYDDLLAKDCHCI

SEQ ID NO: 49 - protein, 98 aa, synthetic construct
CRLHTVRASLEDLGWADWVLSPREVQVTMCIGACPSQFRAANMHAQIKTSLHRLKPDTVPAPCCVPASYNPMVLIQKTDTGVSLQTYDDLLAKDCHCI

SEQ ID NO: 50 - protein, 108 aa, synthetic construct
EHCPLGPGRCCRLHTVRASLEDLGWADWVLSPREVQVTMCIGACPSQFRAANMHAQIKTSLHRLKPDTVPAPCCVPASYNPMVLIQKTDTGVSLQTYDDLLAKDCHCI

SEQ ID NO: 51 - protein, 107 aa, synthetic construct
DCPLGPGRCCRLHTVRASLEDLGWADWVLSPREVQVTMCIGACPSQFRAANMHAQIKTSLHRLKPDTVPAPCCVPASYNPMVLIQKTDTGVSLQTYDDLLAKDCHCI

SEQ ID NO: 52 - protein, 108 aa, synthetic construct
DECPLGPGRCCRLHTVRASLEDLGWADWVLSPREVQVTMCIGACPSQFRAANMHAQIKTSLHRLKPDTVPAPCCVPASYNPMVLIQKTDTGVSLQTYDDLLAKDCHCI

SEQ ID NO: 53 - protein, 107 aa, synthetic construct
ECPLGPGRCCRLHTVRASLEDLGWADWVLSPREVQVTMCIGACPSQFRAANMHAQIKTSLHRLKPDTVPAPCCVPASYNPMVLIQKTDTGVSLQTYDDLLAKDCHCI

SEQ ID NO: 54 - protein, 108 aa, synthetic construct
DHCPLGPGRCCRLHTVQASLEDLGWADWVLSPREVQVTMCIGACPSQFRAANMHAQIKTSLHRLKPDTVPAPCCVPASYNPMVLIQKTDTGVSLQTYDDLLAKDCHCI

SEQ ID NO: 55 - protein, 108 aa, synthetic construct
DHCPLGPGRCCRLHTVHASLEDLGWADWVLSPREVQVTMCIGACPSQFRAANMHAQIKTSLHRLKPDTVPAPCCVPASYNPMVLIQKTDTGVSLQTYDDLLAKDCHCI

SEQ ID NO: 56 - protein, 108 aa, synthetic construct
DHCPLGPGRCCRLHTVRASLEELGWADWVLSPREVQVTMCIGACPSQFRAANMHAQIKTSLHRLKPDTVPAPCCVPASYNPMVLIQKTDTGVSLQTYDDLLAKDCHCI

SEQ ID NO: 57 - protein, 108 aa, synthetic construct
DHCPLGPGRCCRLHTVRASLEELGWADWVLSPREVQVTMCIGACPSQFRAANMHAQIKTSLHRLRPDTVPAPCCVPASYNPMVLIQKTDTGVSLQTYDDLLAKDCHCI

SEQ ID NO: 58 - protein, 108 aa, synthetic construct
DHCPLGPGRCCRLHTVRASLEDLGWSDWVLSPREVQVTMCIGACPSQFRAANMHAQIKTSLHRLKPDTVPAPCCVPASYNPMVLIQKTDTGVSLQTYDDLLAKDCHCI

SEQ ID NO: 59 - protein, 108 aa, synthetic construct
DHCPLGPGRCCRLHTVRASLEDLGWADWVLSPREVQVTMCIGDCPSQFRAANMHAQIKTSLHRLKPDTVPAPCCVPASYNPMVLIQKTDTGVSLQTYDDLLAKDCHCI

SEQ ID NO: 60 - protein, 108 aa, synthetic construct
DHCPLGPGRCCRLHTVRASLEDLGWADWVLSPREVQVTMCIGACPSQFRSANMHAQIKTSLHRLKPDTVPAPCCVPASYNPMVLIQKTDTGVSLQTYDDLLAKDCHCI

SEQ ID NO: 61 - protein, 108 aa, synthetic construct
DHCPLGPGRCCRLHTVRASLEDLGWADWVLSPREVQVTMCIGACPSQFRAENMHAQIKTSLHRLKPDTVPAPCCVPASYNPMVLIQKTDTGVSLQTYDDLLAKDCHCI

SEQ ID NO: 62 - protein, 108 aa, synthetic construct
DHCPLGPGRCCRLHTVRASLEDLGWADWVLSPREVQVTMCIGACPSQFRAANTHAQIKTSLHRLKPDTVPAPCCVPASYNPMVLIQKTDTGVSLQTYDDLLAKDCHCI

SEQ ID NO: 63 - protein, 108 aa, synthetic construct
DHCPLGPGRCCRLHTVRASLEDLGWADWVLSPREVQVTMCIGACPSQFRAANMHAQIKTSLHQLKPDTVPAPCCVPASYNPMVLIQKTDTGVSLQTYDDLLAKDCHCI

SEQ ID NO: 64 - protein, 108 aa, synthetic construct
DHCPLGPGRCCRLHTVRASLEDLGWADWVLSPREVQVTMCIGACPSQFRAANMHAQIKTSLHRLKPDTVPAPCCVPSSYNPMVLIQKTDTGVSLQTYDDLLAKDCHCI

SEQ ID NO: 65 - protein, 108 aa, synthetic construct
DHCPLGPGRCCRLHTVRASLEDLGWADWVLSPREVQVTMCIGACPSQFRAANMHAQIKTSLHRLKPDTVPAPCCVPASYNPMVLIQKTDEGVSLQTYDDLLAKDCHCI

SEQ ID NO: 66 - protein, 108 aa, synthetic construct
DHCPLGPGRCCRLHTVRASLEDLGWADWVLSPREVQVTMCIGACPSQFRAANMHAQIKTSLHRLKPDTVPAPCCVPASYNPMVLIQKTDTGVSLQTYDDLLAQDCHCI

SEQ ID NO: 67 - protein, 368 aa, synthetic construct
APEAAGGPSVFLFPPKPKDTLMISRTPEVTCVVVDVSQEDPEVQFNWYVDGVEVHNAKTKPREEQFNSTYRVVSVLTVLHQDWLNGKEYKCKVSNKGLPSSIEKTISKAKGQPREPQVYTLPPSQEEMTKNQVSLTCLVKGFYPSDIAVEWESNGQPENNYKTTPPVLDSDGSFFLYSRLTVDKSRWQEGNVFSCSVMHEALHNHYTQESLSLSLGGGGGSGGGGSAPAPAPAPAPAPAPAPAPAPGGGGSGGGGSARNGDHCPLGPGRCCRLHTVRASLEDLGWADWVLSPREVQVTMCIGACPSQFRAANMHAQIKTSLHRLKPDTVPAPCCVPASYNPMVLIQKTDTGVSLQTYDDLLAKDCHCI

SEQ ID NO: 68 - protein, 365 aa, synthetic construct
APEAAGGPSVFLFPPKPKDTLMISRTPEVTCVVVDVSQEDPEVQFNWYVDGVEVHNAKTKPREEQFNSTYRVVSVLTVLHQDWLNGKEYKCKVSNKGLPSSIEKTISKAKGQPREPQVYTLPPSQEEMTKNQVSLTCLVKGFYPSDIAVEWESNGQPENNYKTTPPVLDSDGSFFLYSRLTVDKSRWQEGNVFSCSVMHEALHNHYTQESLSLSLGGGGGSGGGGSAPAPAPAPAPAPAPAPAPAPGGGGSGGGGSGDHCPLGPGRCCRLHTVRASLEDLGWADWVLSPREVQVTMCIGACPSQFRAANMHAQIKTSLHRLKPDTVPAPCCVPASYNPMVLIQKTDTGVSLQTYDDLLAKDCHCI

SEQ ID NO: 69 - protein, 364 aa, synthetic construct
APEAAGGPSVFLFPPKPKDTLMISRTPEVTCVVVDVSQEDPEVQFNWYVDGVEVHNAKTKPREEQFNSTYRVVSVLTVLHQDWLNGKEYKCKVSNKGLPSSIEKTISKAKGQPREPQVYTLPPSQEEMTKNQVSLTCLVKGFYPSDIAVEWESNGQPENNYKTTPPVLDSDGSFFLYSRLTVDKSRWQEGNVFSCSVMHEALHNHYTQESLSLSLGGGGGSGGGGSAPAPAPAPAPAPAPAPAPAPGGGGSGGGGSDHCPLGPGRCCRLHTVRASLEDLGWADWVLSPREVQVTMCIGACPSQFRAANMHAQIKTSLHRLKPDTVPAPCCVPASYNPMVLIQKTDTGVSLQTYDDLLAKDCHCI

SEQ ID NO: 70 - protein, 364 aa, synthetic construct
APEAAGGPSVFLFPPKPKDTLMISRTPEVTCVVVDVSQEDPEVQFNWYVDGVEVHNAKTKPREEQFNSTYRVVSVLTVLHQDWLNGKEYKCKVSNKGLPSSIEKTISKAKGQPREPQVYTLPPSQEEMTKNQVSLTCLVKGFYPSDIAVEWESNGQPENNYKTTPPVLDSDGSFFLYSRLTVDKSRWQEGNVFSCSVMHEALHNHYTQDSLSLSLGGGGGSGGGGSAPAPAPAPAPAPAPAPAPAPGGGGSGGGGSDHCPLGPGRCCRLHTVRASLEDLGWADWVLSPREVQVTMCIGACPSQFRAANMHAQIKTSLHRLKPDTVPAPCCVPASYNPMVLIQKTDTGVSLQTYDDLLAKDCHCI

SEQ ID NO: 71 - protein, 364 aa, synthetic construct
APEAAGGPSVFLFPPKPKDTLMISRTPEVTCVVVDVSQEDPEVQFNWYVDGVEVHNAKTKPREEQFNSTYRVVSVLTVLHQDWLNGKEYKCKVSNKGLPSSIEKTISKAKGQPREPQVYTLPPSQEEMTKNQVSLTCLVKGFYPSDIAVEWESNGQPENNYKTTPPVLDSDGSFFLYSRLTVDKSRWQEGNVFSCSVMHEALHNHYTQQSLSLSLGGGGGSGGGGSAPAPAPAPAPAPAPAPAPAPGGGGSGGGGSDHCPLGPGRCCRLHTVRASLEDLGWADWVLSPREVQVTMCIGACPSQFRAANMHAQIKTSLHRLKPDTVPAPCCVPASYNPMVLIQKTDTGVSLQTYDDLLAKDCHCI

SEQ ID NO: 72 - protein, 364 aa, synthetic construct
APEAAGGPSVFLFPPKPKDTLMISRTPEVTCVVVDVSQEDPEVQFNWYVDGVEVHNAKTKPREEQFNSTYRVVSVLTVLHQDWLNGKEYKCKVSNKGLPSSIEKTISKAKGQPREPQVYTLPPSQEEMTKNQVSLTCLVKGFYPSDIAVEWESNGQPENNYKTTPPVLDSDGSFFLYSRLTVDKSRWQEGNVFSCSVMHEALHNHYTQASLSLSLGGGGGSGGGGSAPAPAPAPAPAPAPAPAPAPGGGGSGGGGSDHCPLGPGRCCRLHTVRASLEDLGWADWVLSPREVQVTMCIGACPSQFRAANMHAQIKTSLHRLKPDTVPAPCCVPASYNPMVLIQKTDTGVSLQTYDDLLAKDCHCI

SEQ ID NO: 73 - protein, 364 aa, synthetic construct
APEAAGGPSVFLFPPKPKDTLMISRTPEVTCVVVDVSQEDPEVQFNWYVDGVEVHNAKTKPREEQFNSTYRVVSVLTVLHQDWLNGKEYKCKVSNKGLPSSIEKTISKAKGQPREPQVYTLPPSQKEMTKNQVSLTCLVKGFYPSDIAVEWESNGQPENNYKTTPPVLDSDGSFFLYSRLTVDKSRWQEGNVFSCSVMHEALHNHYTQKSLSLSLGGGGGSGGGGSAPAPAPAPAPAPAPAPAPAPGGGGSGGGGSDHCPLGPGRCCRLHTVRASLEDLGWADWVLSPREVQVTMCIGACPSQFRAANMHAQIKTSLHRLKPDTVPAPCCVPASYNPMVLIQKTDTGVSLQTYDDLLAKDCHCI

SEQ ID NO: 74 - protein, 364 aa, synthetic construct
APEAAGGPSVFLFPPKPKDTLMISRTPEVTCVVVDVSQEDPEVQFNWYVDGVEVHNAKTKPREEQFNSTYRVVSVLTVLHQDWLNGKEYKCKVSNKGLPSSIEKTISKAKGQPREPQVYTLPPSQREMTKNQVSLTCLVKGFYPSDIAVEWESNGQPENNYKTTPPVLDSDGSFFLYSRLTVDKSRWQEGNVFSCSVMHEALHNHYTQKSLSLSLGGGGGSGGGGSAPAPAPAPAPAPAPAPAPAPGGGGSGGGGSDHCPLGPGRCCRLHTVRASLEDLGWADWVLSPREVQVTMCIGACPSQFRAANMHAQIKTSLHRLKPDTVPAPCCVPASYNPMVLIQKTDTGVSLQTYDDLLAKDCHCI

SEQ ID NO: 75 - protein, 364 aa, synthetic construct
APEAAGGPSVFLFPPKPKDTLMISRTPEVTCVVVDVSQEDPEVQFNWYVDGVEVHNAKTKPREEQFNSTYRVVSVLTVLHQDWLNGKEYKCKVSNKGLPSSIEKTISKAKGQPREPQVYTLPPSQQEMTKNQVSLTCLVKGFYPSDIAVEWESNGQPENNYKTTPPVLDSDGSFFLYSRLTVDKSRWQEGNVFSCSVMHEALHNHYTQKSLSLSLGGGGGSGGGGSAPAPAPAPAPAPAPAPAPAPGGGGSGGGGSDHCPLGPGRCCRLHTVRASLEDLGWADWVLSPREVQVTMCIGACPSQFRAANMHAQIKTSLHRLKPDTVPAPCCVPASYNPMVLIQKTDTGVSLQTYDDLLAKDCHCI

SEQ ID NO: 76 - protein, 364 aa, synthetic construct
APEAAGGPSVFLFPPKPKDTLMISRTPEVTCVVVDVSQEDPEVQFNWYVDGVEVHNAKTKPREEQFNSTYRVVSVLTVLHQDWLNGKEYKCKVSNKGLPSSIEKTISKAKGQPREPQVYTLPPSQAEMTKNQVSLTCLVKGFYPSDIAVEWESNGQPENNYKTTPPVLDSDGSFFLYSRLTVDKSRWQEGNVFSCSVMHEALHNHYTQKSLSLSLGGGGGSGGGGSAPAPAPAPAPAPAPAPAPAPGGGGSGGGGSDHCPLGPGRCCRLHTVRASLEDLGWADWVLSPREVQVTMCIGACPSQFRAANMHAQIKTSLHRLKPDTVPAPCCVPASYNPMVLIQKTDTGVSLQTYDDLLAKDCHCI

SEQ ID NO: 77 - protein, 364 aa, synthetic construct
APEAAGGPSVFLFPPKPKDTLMISRTPEVTCVVVDVSHEDPEVKFNWYVDGVEVHNAKTKPREEQYNSTYRVVSVLTVLHQDWLNGKEYKCKVSNKALPAPIEKTISKAKGQPREPQVYTLPPSRDELTKNQVSLTCLVKGFYPSDIAVEWESNGQPENNYKTTPPVLDSDGSFFLYSKLTVDKSRWQQGNVFSCSVMHEALHNHYTQESLSLSPGGGGGSGGGGSAPAPAPAPAPAPAPAPAPAPGGGGSGGGGSDHCPLGPGRCCRLHTVRASLEDLGWADWVLSPREVQVTMCIGACPSQFRAANMHAQIKTSLHRLKPDTVPAPCCVPASYNPMVLIQKTDTGVSLQTYDDLLAKDCHCI

SEQ ID NO: 78 - protein, 362 aa, synthetic construct
EAAGGPSVFLFPPKPKDTLMISRTPEVTCVVVDVSQEDPEVQFNWYVDGVEVHNAKTKPREEQFNSTYRVVSVLTVLHQDWLNGKEYKCKVSNKGLPSSIEKTISKAKGQPREPQVYTLPPSQEEMTKNQVSLTCLVKGFYPSDIAVEWESNGQPENNYKTTPPVLDSDGSFFLYSRLTVDKSRWQEGNVFSCSVMHEALHNHYTQESLSLSLGGGGGSGGGGSAPAPAPAPAPAPAPAPAPAPGGGGSGGGGSDHCPLGPGRCCRLHTVRASLEDLGWADWVLSPREVQVTMCIGACPSQFRAANMHAQIKTSLHRLKPDTVPAPCCVPASYNPMVLIQKTDTGVSLQTYDDLLAKDCHCI

SEQ ID NO: 79 - protein, 359 aa, synthetic construct
GGPSVFLFPPKPKDTLMISRTPEVTCVVVDVSQEDPEVQFNWYVDGVEVHNAKTKPREEQFNSTYRVVSVLTVLHQDWLNGKEYKCKVSNKGLPSSIEKTISKAKGQPREPQVYTLPPSQEEMTKNQVSLTCLVKGFYPSDIAVEWESNGQPENNYKTTPPVLDSDGSFFLYSRLTVDKSRWQEGNVFSCSVMHEALHNHYTQKSLSLSLGGGGGSGGGGSAPAPAPAPAPAPAPAPAPAPGGGGSGGGGSDHCPLGPGRCCRLHTVRASLEDLGWADWVLSPREVQVTMCIGACPSQFRAANMHAQIKTSLHRLKPDTVPAPCCVPASYNPMVLIQKTDTGVSLQTYDDLLAKDCHCI

SEQ ID NO: 80 - protein, 359 aa, synthetic construct
GGPSVFLFPPKPKDTLMISRTPEVTCVVVDVSQEDPEVQFNWYVDGVEVHNAKTKPREEQFNSTYRVVSVLTVLHQDWLNGKEYKCKVSNKGLPSSIEKTISKAKGQPREPQVYTLPPSQEEMTKNQVSLTCLVKGFYPSDIAVEWESNGQPENNYKTTPPVLDSDGSFFLYSRLTVDKSRWQEGNVFSCSVMHEALHNHYTQESLSLSLGGGGGSGGGGSAPAPAPAPAPAPAPAPAPAPGGGGSGGGGSDHCPLGPGRCCRLHTVRASLEDLGWADWVLSPREVQVTMCIGACPSQFRAANMHAQIKTSLHRLKPDTVPAPCCVPASYNPMVLIQKTDTGVSLQTYDDLLAKDCHCI

SEQ ID NO: 81 - protein, 358 aa, synthetic construct
GPSVFLFPPKPKDTLMISRTPEVTCVVVDVSQEDPEVQFNWYVDGVEVHNAKTKPREEQFNSTYRVVSVLTVLHQDWLNGKEYKCKVSNKGLPSSIEKTISKAKGQPREPQVYTLPPSQEEMTKNQVSLTCLVKGFYPSDIAVEWESNGQPENNYKTTPPVLDSDGSFFLYSRLTVDKSRWQEGNVFSCSVMHEALHNHYTQESLSLSLGGGGGSGGGGSAPAPAPAPAPAPAPAPAPAPGGGGSGGGGSDHCPLGPGRCCRLHTVRASLEDLGWADWVLSPREVQVTMCIGACPSQFRAANMHAQIKTSLHRLKPDTVPAPCCVPASYNPMVLIQKTDTGVSLQTYDDLLAKDCHCI

SEQ ID NO: 82 - protein, 348 aa, synthetic construct
GGPSVFLFPPKPKDTLMISRTPEVTCVVVDVSQEDPEVQFNWYVDGVEVHNAKTKPREEQFNSTYRVVSVLTVLHQDWLNGKEYKCKVSNKGLPSSIEKTISKAKGQPREPQVYTLPPSQEEMTKNQVSLTCLVKGFYPSDIAVEWESNGQPENNYKTTPPVLDSDGSFFLYSRLTVDKSRWQEGNVFSCSVMHEALHNHYTQESLSLSLGGGGGAPAPAPAPAPAPAPAPAPAPGGGGGDHCPLGPGRCCRLHTVRASLEDLGWADWVLSPREVQVTMCIGACPSQFRAANMHAQIKTSLHRLKPDTVPAPCCVPASYNPMVLIQKTDTGVSLQTYDDLLAKDCHCI

SEQ ID NO: 83 - protein, 359 aa, synthetic construct
GGPSVFLFPPKPKDTLMISRTPEVTCVVVDVSQEDPEVQFNWYVDGVEVHNAKTKPREEQFNSTYRVVSVLTVLHQDWLNGKEYKCKVSNKGLPSSIEKTISKAKGQPREPQVYTLPPSQEEMTKNQVSLTCLVKGFYPSDIAVEWESNGQPENNYKTTPPVLDSDGSFFLYSRLTVDKSRWQEGNVFSCSVMHEALHNHYTQESLSLSLGGGGGSGGGGSEPEPEPEPEPEPEPEPEPEPGGGGSGGGGSDHCPLGPGRCCRLHTVRASLEDLGWADWVLSPREVQVTMCIGACPSQFRAANMHAQIKTSLHRLKPDTVPAPCCVPASYNPMVLIQKTDTGVSLQTYDDLLAKDCHCI

SEQ ID NO: 84 - protein, 359 aa, synthetic construct
GGPSVFLFPPKPKDTLMISRTPEVTCVVVDVSQEDPEVQFNWYVDGVEVHNAKTKPREEQFNSTYRVVSVLTVLHQDWLNGKEYKCKVSNKGLPSSIEKTISKAKGQPREPQVYTLPPSQEEMTKNQVSLTCLVKGFYPSDIAVEWESNGQPENNYKTTPPVLDSDGSFFLYSRLTVDKSRWQEGNVFSCSVMHEALHNHYTQESLSLSLGGGGGSGGGGSGGGGSGGGGSGGGGSGGGGSGGGGSGGGGSDHCPLGPGRCCRLHTVRASLEDLGWADWVLSPREVQVTMCIGACPSQFRAANMHAQIKTSLHRLKPDTVPAPCCVPASYNPMVLIQKTDTGVSLQTYDDLLAKDCHCI

SEQ ID NO: 85 - protein, 364 aa, synthetic construct
APEAAGGPSVFLFPPKPKDTLMISRTPEVTCVVVDVSQEDPEVQFNWYVDGVEVHNAKTKPREEQFNSTYRVVSVLTVLHQDWLNGKEYKCKVSNKGLPSSIEKTISKAKGQPREPQVYTLPPSQEEMTKNQVSLTCLVKGFYPSDIAVEWESNGQPENNYKTTPPVLDSDGSFFLYSRLTVDKSRWQEGNVFSCSVMHEALHNHYTQESLSLSLGGGGGSGGGGSAPAPAPAPAPAPAPAPAPAPGGGGSGGGGSEHCPLGPGRCCRLHTVRASLEDLGWADWVLSPREVQVTMCIGACPSQFRAANMHAQIKTSLHRLKPDTVPAPCCVPASYNPMVLIQKTDTGVSLQTYDDLLAKDCHCI

SEQ ID NO: 86 - protein, 363 aa, synthetic construct
APEAAGGPSVFLFPPKPKDTLMISRTPEVTCVVVDVSQEDPEVQFNWYVDGVEVHNAKTKPREEQFNSTYRVVSVLTVLHQDWLNGKEYKCKVSNKGLPSSIEKTISKAKGQPREPQVYTLPPSQEEMTKNQVSLTCLVKGFYPSDIAVEWESNGQPENNYKTTPPVLDSDGSFFLYSRLTVDKSRWQEGNVFSCSVMHEALHNHYTQESLSLSLGGGGGSGGGGSAPAPAPAPAPAPAPAPAPAPGGGGSGGGGSDCPLGPGRCCRLHTVRASLEDLGWADWVLSPREVQVTMCIGACPSQFRAANMHAQIKTSLHRLKPDTVPAPCCVPASYNPMVLIQKTDTGVSLQTYDDLLAKDCHCI

SEQ ID NO: 87 - protein, 364 aa, synthetic construct
APEAAGGPSVFLFPPKPKDTLMISRTPEVTCVVVDVSQEDPEVQFNWYVDGVEVHNAKTKPREEQFNSTYRVVSVLTVLHQDWLNGKEYKCKVSNKGLPSSIEKTISKAKGQPREPQVYTLPPSQEEMTKNQVSLTCLVKGFYPSDIAVEWESNGQPENNYKTTPPVLDSDGSFFLYSRLTVDKSRWQEGNVFSCSVMHEALHNHYTQESLSLSLGGGGGSGGGGSAPAPAPAPAPAPAPAPAPAPGGGGSGGGGSDECPLGPGRCCRLHTVRASLEDLGWADWVLSPREVQVTMCIGACPSQFRAANMHAQIKTSLHRLKPDTVPAPCCVPASYNPMVLIQKTDTGVSLQTYDDLLAKDCHCI

SEQ ID NO: 88 - protein, 363 aa, synthetic construct
APEAAGGPSVFLFPPKPKDTLMISRTPEVTCVVVDVSQEDPEVQFNWYVDGVEVHNAKTKPREEQFNSTYRVVSVLTVLHQDWLNGKEYKCKVSNKGLPSSIEKTISKAKGQPREPQVYTLPPSQEEMTKNQVSLTCLVKGFYPSDIAVEWESNGQPENNYKTTPPVLDSDGSFFLYSRLTVDKSRWQEGNVFSCSVMHEALHNHYTQESLSLSLGGGGGSGGGGSAPAPAPAPAPAPAPAPAPAPGGGGSGGGGSECPLGPGRCCRLHTVRASLEDLGWADWVLSPREVQVTMCIGACPSQFRAANMHAQIKTSLHRLKPDTVPAPCCVPASYNPMVLIQKTDTGVSLQTYDDLLAKDCHCI

SEQ ID NO: 89 - protein, 364 aa, synthetic construct
APEAAGGPSVFLFPPKPKDTLMISRTPEVTCVVVDVSQEDPEVQFNWYVDGVEVHNAKTKPREEQFNSTYRVVSVLTVLHQDWLNGKEYKCKVSNKGLPSSIEKTISKAKGQPREPQVYTLPPSQEEMTKNQVSLTCLVKGFYPSDIAVEWESNGQPENNYKTTPPVLDSDGSFFLYSRLTVDKSRWQEGNVFSCSVMHEALHNHYTQESLSLSLGGGGGSGGGGSAPAPAPAPAPAPAPAPAPAPGGGGSGGGGSDHCPLGPGRCCRLHTVQASLEDLGWADWVLSPREVQVTMCIGACPSQFRAANMHAQIKTSLHRLKPDTVPAPCCVPASYNPMVLIQKTDTGVSLQTYDDLLAKDCHCI

SEQ ID NO: 90 - protein, 364 aa, synthetic construct
APEAAGGPSVFLFPPKPKDTLMISRTPEVTCVVVDVSQEDPEVQFNWYVDGVEVHNAKTKPREEQFNSTYRVVSVLTVLHQDWLNGKEYKCKVSNKGLPSSIEKTISKAKGQPREPQVYTLPPSQEEMTKNQVSLTCLVKGFYPSDIAVEWESNGQPENNYKTTPPVLDSDGSFFLYSRLTVDKSRWQEGNVFSCSVMHEALHNHYTQESLSLSLGGGGGSGGGGSAPAPAPAPAPAPAPAPAPAPGGGGSGGGGSDHCPLGPGRCCRLHTVHASLEDLGWADWVLSPREVQVTMCIGACPSQFRAANMHAQIKTSLHRLKPDTVPAPCCVPASYNPMVLIQKTDTGVSLQTYDDLLAKDCHCI

SEQ ID NO: 91 - protein, 364 aa, synthetic construct
APEAAGGPSVFLFPPKPKDTLMISRTPEVTCVVVDVSQEDPEVQFNWYVDGVEVHNAKTKPREEQFNSTYRVVSVLTVLHQDWLNGKEYKCKVSNKGLPSSIEKTISKAKGQPREPQVYTLPPSQEEMTKNQVSLTCLVKGFYPSDIAVEWESNGQPENNYKTTPPVLDSDGSFFLYSRLTVDKSRWQEGNVFSCSVMHEALHNHYTQESLSLSLGGGGGSGGGGSAPAPAPAPAPAPAPAPAPAPGGGGSGGGGSDHCPLGPGRCCRLHTVRASLEELGWADWVLSPREVQVTMCIGACPSQFRAANMHAQIKTSLHRLKPDTVPAPCCVPASYNPMVLIQKTDTGVSLQTYDDLLAKDCHCI

SEQ ID NO: 92 - protein, 364 aa, synthetic construct
APEAAGGPSVFLFPPKPKDTLMISRTPEVTCVVVDVSQEDPEVQFNWYVDGVEVHNAKTKPREEQFNSTYRVVSVLTVLHQDWLNGKEYKCKVSNKGLPSSIEKTISKAKGQPREPQVYTLPPSQEEMTKNQVSLTCLVKGFYPSDIAVEWESNGQPENNYKTTPPVLDSDGSFFLYSRLTVDKSRWQEGNVFSCSVMHEALHNHYTQESLSLSLGGGGGSGGGGSAPAPAPAPAPAPAPAPAPAPGGGGSGGGGSDHCPLGPGRCCRLHTVRASLEELGWADWVLSPREVQVTMCIGACPSQFRAANMHAQIKTSLHRLRPDTVPAPCCVPASYNPMVLIQKTDTGVSLQTYDDLLAKDCHCI

SEQ ID NO: 93 - protein, 364 aa, synthetic construct; identical to SEQ ID NO: 69

SEQ ID NO: 94 - protein, 364 aa, synthetic construct
APEAAGGPSVFLFPPKPKDTLMISRTPEVTCVVVDVSQEDPEVQFNWYVDGVEVHNAKTKPREEQFNSTYRVVSVLTVLHQDWLNGKEYKCKVSNKGLPSSIEKTISKAKGQPREPQVYTLPPSQEEMTKNQVSLTCLVKGFYPSDIAVEWESNGQPENNYKTTPPVLDSDGSFFLYSRLTVDKSRWQEGNVFSCSVMHEALHNHYTQESLSLSLGGGGGSGGGGSAPAPAPAPAPAPAPAPAPAPGGGGSGGGGSDHCPLGPGRCCRLHTVRASLEDLGWADWVLSPREVQVTMCIGDCPSQFRAANMHAQIKTSLHRLKPDTVPAPCCVPASYNPMVLIQKTDTGVSLQTYDDLLAKDCHCI

SEQ ID NO: 95 - protein, 364 aa, synthetic construct
APEAAGGPSVFLFPPKPKDTLMISRTPEVTCVVVDVSQEDPEVQFNWYVDGVEVHNAKTKPREEQFNSTYRVVSVLTVLHQDWLNGKEYKCKVSNKGLPSSIEKTISKAKGQPREPQVYTLPPSQEEMTKNQVSLTCLVKGFYPSDIAVEWESNGQPENNYKTTPPVLDSDGSFFLYSRLTVDKSRWQEGNVFSCSVMHEALHNHYTQESLSLSLGGGGGSGGGGSAPAPAPAPAPAPAPAPAPAPGGGGSGGGGSDHCPLGPGRCCRLHTVRASLEDLGWADWVLSPREVQVTMCIGACPSQFRSANMHAQIKTSLHRLKPDTVPAPCCVPASYNPMVLIQKTDTGVSLQTYDDLLAKDCHCI

SEQ ID NO: 96 - protein, 364 aa, synthetic construct
APEAAGGPSVFLFPPKPKDTLMISRTPEVTCVVVDVSQEDPEVQFNWYVDGVEVHNAKTKPREEQFNSTYRVVSVLTVLHQDWLNGKEYKCKVSNKGLPSSIEKTISKAKGQPREPQVYTLPPSQEEMTKNQVSLTCLVKGFYPSDIAVEWESNGQPENNYKTTPPVLDSDGSFFLYSRLTVDKSRWQEGNVFSCSVMHEALHNHYTQESLSLSLGGGGGSGGGGSAPAPAPAPAPAPAPAPAPAPGGGGSGGGGSDHCPLGPGRCCRLHTVRASLEDLGWADWVLSPREVQVTMCIGACPSQFRAENMHAQIKTSLHRLKPDTVPAPCCVPASYNPMVLIQKTDTGVSLQTYDDLLAKDCHCI

SEQ ID NO: 97 - protein, 364 aa, synthetic construct
APEAAGGPSVFLFPPKPKDTLMISRTPEVTCVVVDVSQEDPEVQFNWYVDGVEVHNAKTKPREEQFNSTYRVVSVLTVLHQDWLNGKEYKCKVSNKGLPSSIEKTISKAKGQPREPQVYTLPPSQEEMTKNQVSLTCLVKGFYPSDIAVEWESNGQPENNYKTTPPVLDSDGSFFLYSRLTVDKSRWQEGNVFSCSVMHEALHNHYTQESLSLSLGGGGGSGGGGSAPAPAPAPAPAPAPAPAPAPGGGGSGGGGSDHCPLGPGRCCRLHTVRASLEDLGWADWVLSPREVQVTMCIGACPSQFRAANTHAQIKTSLHRLKPDTVPAPCCVPASYNPMVLIQKTDTGVSLQTYDDLLAKDCHCI

SEQ ID NO: 98 - protein, 364 aa, synthetic construct
APEAAGGPSVFLFPPKPKDTLMISRTPEVTCVVVDVSQEDPEVQFNWYVDGVEVHNAKTKPREEQFNSTYRVVSVLTVLHQDWLNGKEYKCKVSNKGLPSSIEKTISKAKGQPREPQVYTLPPSQEEMTKNQVSLTCLVKGFYPSDIAVEWESNGQPENNYKTTPPVLDSDGSFFLYSRLTVDKSRWQEGNVFSCSVMHEALHNHYTQESLSLSLGGGGGSGGGGSAPAPAPAPAPAPAPAPAPAPGGGGSGGGGSDHCPLGPGRCCRLHTVRASLEDLGWADWVLSPREVQVTMCIGACPSQFRAANMHAQIKTSLHQLKPDTVPAPCCVPASYNPMVLIQKTDTGVSLQTYDDLLAKDCHCI

SEQ ID NO: 99 - protein, 364 aa, synthetic construct
APEAAGGPSVFLFPPKPKDTLMISRTPEVTCVVVDVSQEDPEVQFNWYVDGVEVHNAKTKPREEQFNSTYRVVSVLTVLHQDWLNGKEYKCKVSNKGLPSSIEKTISKAKGQPREPQVYTLPPSQEEMTKNQVSLTCLVKGFYPSDIAVEWESNGQPENNYKTTPPVLDSDGSFFLYSRLTVDKSRWQEGNVFSCSVMHEALHNHYTQESLSLSLGGGGGSGGGGSAPAPAPAPAPAPAPAPAPAPGGGGSGGGGSDHCPLGPGRCCRLHTVRASLEDLGWADWVLSPREVQVTMCIGACPSQFRAANMHAQIKTSLHRLKPDTVPAPCCVPSSYNPMVLIQKTDTGVSLQTYDDLLAKDCHCI

SEQ ID NO: 100 - protein, 364 aa, synthetic construct
APEAAGGPSVFLFPPKPKDTLMISRTPEVTCVVVDVSQEDPEVQFNWYVDGVEVHNAKTKPREEQFNSTYRVVSVLTVLHQDWLNGKEYKCKVSNKGLPSSIEKTISKAKGQPREPQVYTLPPSQEEMTKNQVSLTCLVKGFYPSDIAVEWESNGQPENNYKTTPPVLDSDGSFFLYSRLTVDKSRWQEGNVFSCSVMHEALHNHYTQESLSLSLGGGGGSGGGGSAPAPAPAPAPAPAPAPAPAPGGGGSGGGGSDHCPLGPGRCCRLHTVRASLEDLGWADWVLSPREVQVTMCIGACPSQFRAANMHAQIKTSLHRLKPDTVPAPCCVPASYNPMVLIQKTDEGVSLQTYDDLLAKDCHCI

SEQ ID NO: 101 - protein, 364 aa, synthetic construct
APEAAGGPSVFLFPPKPKDTLMISRTPEVTCVVVDVSQEDPEVQFNWYVDGVEVHNAKTKPREEQFNSTYRVVSVLTVLHQDWLNGKEYKCKVSNKGLPSSIEKTISKAKGQPREPQVYTLPPSQEEMTKNQVSLTCLVKGFYPSDIAVEWESNGQPENNYKTTPPVLDSDGSFFLYSRLTVDKSRWQEGNVFSCSVMHEALHNHYTQESLSLSLGGGGGSGGGGSAPAPAPAPAPAPAPAPAPAPGGGGSGGGGSDHCPLGPGRCCRLHTVRASLEDLGWADWVLSPREVQVTMCIGACPSQFRAANMHAQIKTSLHRLKPDTVPAPCCVPASYNPMVLIQKTDTGVSLQTYDDLLAQDCHCI

SEQ ID NO: 102 - protein, 354 aa, synthetic construct
APEAAGGPSVFLFPPKPKDTLMISRTPEVTCVVVDVSQEDPEVQFNWYVDGVEVHNAKTKPREEQFNSTYRVVSVLTVLHQDWLNGKEYKCKVSNKGLPSSIEKTISKAKGQPREPQVYTLPPSQEEMTKNQVSLTCLVKGFYPSDIAVEWESNGQPENNYKTTPPVLDSDGSFFLYSRLTVDKSRWQEGNVFSCSVMHEALHNHYTQESLSLSLGGGGGSGGGGSAPAPAPAPAPAPAPAPAPAPGGGGSGGGGSCRLHTVRASLEDLGWADWVLSPREVQVTMCIGACPSQFRAANMHAQIKTSLHRLKPDTVPAPCCVPASYNPMVLIQKTDTGVSLQTYDDLLAKDCHCI

SEQ ID NO: 103 - protein, 348 aa, synthetic construct
GGPSVFLFPPKPKDTLMISRTPEVTCVVVDVSQEDPEVQFNWYVDGVEVHNAKTKPREEQFNSTYRVVSVLTVLHQDWLNGKEYKCKVSNKGLPSSIEKTISKAKGQPREPQVYTLPPSQEEMTKNQVSLTCLVKGFYPSDIAVEWESNGQPENNYKTTPPVLDSDGSFQLESRLTVDKSRWQEGNVFSCSVMHEALHNHYTQESLSLSLGGGGGAPAPAPAPAPAPAPAPAPAPGGGGGDHCPLGPGRCCRLHTVRASLEDLGWADWVLSPREVQVTMCIGACPSQFRAANMHAQIKTSLHRLKPDTVPAPCCVPASYNPMVLIQKTDTGVSLQTYDDLLAKDCHCI

SEQ ID NO: 104 - protein, 351 aa, synthetic construct
EAAGGPSVFLFPPKPKDTLMISRTPEVTCVVVDVSQEDPEVQFNWYVDGVEVHNAKTKPREEQFNSTYRVVSVLTVLHQDWLNGKEYKCKVSNKGLPSSIEKTISKAKGQPREPQVYTLPPSQEEMTKNQVSLTCLVKGFYPSDIAVEWESNGQPENNYKTTPPVLDSDGSFQLESRLTVDKSRWQEGNVFSCSVMHEALHNHYTQKSLSLSLGGGGGAPAPAPAPAPAPAPAPAPAPGGGGGDHCPLGPGRCCRLHTVRASLEDLGWADWVLSPREVQVTMCIGACPSQFRAANMHAQIKTSLHRLKPDTVPAPCCVPASYNPMVLIQKTDTGVSLQTYDDLLAKDCHCI

SEQ ID NO: 105 - protein, 365 aa, synthetic construct
APEAAGGPSVFLFPPKPKDTLMISRTPEVTCVVVDVSQEDPEVQFNWYVDGVEVHNAKTKPREEQFNSTYRVVSVLTVLHQDWLNGKEYKCKVSNKGLPSSIEKTISKAKGQPREPQVYTLPPSQEEMTKNQVSLTCLVKGFYPSDIAVEWESNGQPENNYKTTPPVLDSDGSFFLYSRLTVDKSRWQEGNVFSCSVMHEALHNHYTQQSLSLSLGGGGGSGGGGSAPAPAPAPAPAPAPAPAPAPGGGGSGGGGSGDHCPLGPGRCCRLHTVRASLEDLGWADWVLSPREVQVTMCIGACPSQFRAANMHAQIKTSLHRLKPDTVPAPCCVPASYNPMVLIQKTDTGVSLQTYDDLLAKDCHCI

SEQ ID NO: 106 - protein, 365 aa, synthetic construct
APEAAGGPSVFLFPPKPKDTLMISRTPEVTCVVVDVSQEDPEVQFNWYVDGVEVHNAKTKPREEQFNSTYRVVSVLTVLHQDWLNGKEYKCKVSNKGLPSSIEKTISKAKGQPREPQVYTLPPSQQEMTKNQVSLTCLVKGFYPSDIAVEWESNGQPENNYKTTPPVLDSDGSFFLYSRLTVDKSRWQEGNVFSCSVMHEALHNHYTQKSLSLSLGGGGGSGGGGSAPAPAPAPAPAPAPAPAPAPGGGGSGGGGSGDHCPLGPGRCCRLHTVRASLEDLGWADWVLSPREVQVTMCIGACPSQFRAANMHAQIKTSLHRLKPDTVPAPCCVPASYNPMVLIQKTDTGVSLQTYDDLLAKDCHCI

SEQ ID NO: 107 - protein, 365 aa, synthetic construct
APEAAGGPSVFLFPPKPKDTLMISRTPEVTCVVVDVSQEDPEVQFNWYVDGVEVHNAKTKPREEQFNSTYRVVSVLTVLHQDWLNGKEYKCKVSNKGLPSSIEKTISKAKGQPREPQVYTLPPSQEEMTKNQVSLTCLVKGFYPSDIAVEWESNGQPENNYKTTPPVLDSDGSFFLYSRLTVDKSRWQEGNVFSCSVMHEALHNHYTQNSLSLSLGGGGGSGGGGSAPAPAPAPAPAPAPAPAPAPGGGGSGGGGSGDHCPLGPGRCCRLHTVRASLEDLGWADWVLSPREVQVTMCIGACPSQFRAANMHAQIKTSLHRLKPDTVPAPCCVPASYNPMVLIQKTDTGVSLQTYDDLLAKDCHCI

SEQ ID NO: 108 - protein, 365 aa, synthetic construct
APEAAGGPSVFLFPPKPKDTLMISRTPEVTCVVVDVSQEDPEVQFNWYVDGVEVHNAKTKPREEQFNSTYRVVSVLTVLHQDWLNGKEYKCKVSNKGLPSSIEKTISKAKGQPREPQVYTLPPSQNEMTKNQVSLTCLVKGFYPSDIAVEWESNGQPENNYKTTPPVLDSDGSFFLYSRLTVDKSRWQEGNVFSCSVMHEALHNHYTQKSLSLSLGGGGGSGGGGSAPAPAPAPAPAPAPAPAPAPGGGGSGGGGSGDHCPLGPGRCCRLHTVRASLEDLGWADWVLSPREVQVTMCIGACPSQFRAANMHAQIKTSLHRLKPDTVPAPCCVPASYNPMVLIQKTDTGVSLQTYDDLLAKDCHCI

SEQ ID NO: 109 - protein, 365 aa, synthetic construct
APEAAGGPSVFLFPPKPKDTLMISRTPEVTCVVVDVSQEDPEVQFNWYVDGVEVHNAKTKPREEQFNSTYRVVSVLTVLHQDWLNGKEYKCKVSNKGLPSSIEKTISKAKGQPREPQVYTLPPSQEEMTKNQVSLTCLVKGFYPSDIAVEWESNGQPENNYKTTPPVLDSDGSFFLYSRLTVDKSRWQEGNVFSCSVMHEALHNHYTQASLSLSLGGGGGSGGGGSAPAPAPAPAPAPAPAPAPAPGGGGSGGGGSGDHCPLGPGRCCRLHTVRASLEDLGWADWVLSPREVQVTMCIGACPSQFRAANMHAQIKTSLHRLKPDTVPAPCCVPASYNPMVLIQKTDTGVSLQTYDDLLAKDCHCI

SEQ ID NO: 110 - protein, 365 aa, synthetic construct
APEAAGGPSVFLFPPKPKDTLMISRTPEVTCVVVDVSQEDPEVQFNWYVDGVEVHNAKTKPREEQFNSTYRVVSVLTVLHQDWLNGKEYKCKVSNKGLPSSIEKTISKAKGQPREPQVYTLPPSQAEMTKNQVSLTCLVKGFYPSDIAVEWESNGQPENNYKTTPPVLDSDGSFFLYSRLTVDKSRWQEGNVFSCSVMHEALHNHYTQKSLSLSLGGGGGSGGGGSAPAPAPAPAPAPAPAPAPAPGGGGSGGGGSGDHCPLGPGRCCRLHTVRASLEDLGWADWVLSPREVQVTMCIGACPSQFRAANMHAQIKTSLHRLKPDTVPAPCCVPASYNPMVLIQKTDTGVSLQTYDDLLAKDCHCI

SEQ ID NO: 111 - protein, 363 aa, synthetic construct
APEAAGGPSVFLFPPKPKDTLMISRTPEVTCVVVDVSQEDPEVQFNWYVDGVEVHNAKTKPREEQFNSTYRVVSVLTVLHQDWLNGKEYKCKVSNKGLPSSIEKTISKAKGQPREPQVYTLPPSQEEMTKNQVSLTCLVKGFYPSDIAVEWESNGQPENNYKTTPPVLDSDGSFFLYSRLTVDKSRWQEGNVFSCSVMHEALHNHYTQQSLSLSLGGGGGAGGGGAPAPAPAPAPAPAPAPAPAPGGGGAGGGGGDHCPLGPGRCCRLHTVRASLEDLGWADWVLSPREVQVTMCIGACPSQFRAANMHAQIKTSLHRLKPDTVPAPCCVPASYNPMVLIQKTDTGVSLQTYDDLLAKDCHCI

SEQ ID NO: 112 - protein, 363 aa, synthetic construct
APEAAGGPSVFLFPPKPKDTLMISRTPEVTCVVVDVSQEDPEVQFNWYVDGVEVHNAKTKPREEQFNSTYRVVSVLTVLHQDWLNGKEYKCKVSNKGLPSSIEKTISKAKGQPREPQVYTLPPSQEEMTKNQVSLTCLVKGFYPSDIAVEWESNGQPENNYKTTPPVLDSDGSFFLYSRLTVDKSRWQEGNVFSCSVMHEALHNHYTQESLSLSLGGGGGAGGGGAPAPAPAPAPAPAPAPAPAPGGGGAGGGGGDHCPLGPGRCCRLHTVRASLEDLGWADWVLSPREVQVTMCIGACPSQFRAANMHAQIKTSLHRLKPDTVPAPCCVPASYNPMVLIQKTDTGVSLQTYDDLLAKDCHCI

SEQ ID NO: 113 - protein, 365 aa, synthetic construct
APEAAGGPSVFLFPPKPKDTLMISRTPEVTCVVVDVSQEDPEVQFNWYVDGVEVHNAKTKPREEQFNSTYRVVSVLTVLHQDWLNGKEYKCKVSNKGLPSSIEKTISKAKGQPREPQVYTLPPSQEEMTKNQVSLTCLVKGFYPSDIAVEWESNGQPENNYKTTPPVLDSDGSFFLYSRLTVDKSRWQEGNVFSCSVMHEALHNHYTQDSLSLSLGGGGGSGGGGSAPAPAPAPAPAPAPAPAPAPGGGGSGGGGSGDHCPLGPGRCCRLHTVRASLEDLGWADWVLSPREVQVTMCIGACPSQFRAANMHAQIKTSLHRLKPDTVPAPCCVPASYNPMVLIQKTDTGVSLQTYDDLLAKDCHCI

SEQ ID NO: 114 - protein, 365 aa, synthetic construct
APEAAGGPSVFLFPPKPKDTLMISRTPEVTCVVVDVSQEDPEVQFNWYVDGVEVHNAKTKPREEQFNSTYRVVSVLTVLHQDWLNGKEYKCKVSNKGLPSSIEKTISKAKGQPREPQVYTLPPSQKEMTKNQVSLTCLVKGFYPSDIAVEWESNGQPENNYKTTPPVLDSDGSFFLYSRLTVDKSRWQEGNVFSCSVMHEALHNHYTQKSLSLSLGGGGGSGGGGSAPAPAPAPAPAPAPAPAPAPGGGGSGGGGSGDHCPLGPGRCCRLHTVRASLEDLGWADWVLSPREVQVTMCIGACPSQFRAANMHAQIKTSLHRLKPDTVPAPCCVPASYNPMVLIQKTDTGVSLQTYDDLLAKDCHCI

SEQ ID NO: 115 - protein, 365 aa, synthetic construct
APEAAGGPSVFLFPPKPKDTLMISRTPEVTCVVVDVSQEDPEVQFNWYVDGVEVHNAKTKPREEQFNSTYRVVSVLTVLHQDWLNGKEYKCKVSNKGLPSSIEKTISKAKGQPREPQVYTLPPSQREMTKNQVSLTCLVKGFYPSDIAVEWESNGQPENNYKTTPPVLDSDGSFFLYSRLTVDKSRWQEGNVFSCSVMHEALHNHYTQKSLSLSLGGGGGSGGGGSAPAPAPAPAPAPAPAPAPAPGGGGSGGGGSGDHCPLGPGRCCRLHTVRASLEDLGWADWVLSPREVQVTMCIGACPSQFRAANMHAQIKTSLHRLKPDTVPAPCCVPASYNPMVLIQKTDTGVSLQTYDDLLAKDCHCI

SEQ ID NO: 116 - protein, 365 aa, synthetic construct
APEAAGGPSVFLFPPKPKDTLMISRTPEVTCVVVDVSQEDPEVQFNWYVDGVEVHNAKTKPREEQFNSTYRVVSVLTVLHQDWLNGKEYKCKVSNKGLPSSIEKTISKAKGQPREPQVYTLPPSQQEMTKNQVSLTCLVKGFYPSDIAVEWESNGQPENNYKTTPPVLDSDGSFFLYSRLTVDKSRWQEGNVFSCSVMHEALHNHYTQQSLSLSLGGGGGSGGGGSAPAPAPAPAPAPAPAPAPAPGGGGSGGGGSGDHCPLGPGRCCRLHTVRASLEDLGWADWVLSPREVQVTMCIGACPSQFRAANMHAQIKTSLHRLKPDTVPAPCCVPASYNPMVLIQKTDTGVSLQTYDDLLAKDCHCI

SEQ ID NO: 117 - protein, 364 aa, synthetic construct
APEAAGGPSVFLFPPKPKDTLMISRTPEVTCVVVDVSQEDPEVQFNWYVDGVEVHNAKTKPREEQFNSTYRVVSVLTVLHQDWLNGKEYKCKVSNKGLPSSIEKTISKAKGQPREPQVYTLPPSQEEMTKNQVSLTCLVKGFYPSDIAVEWESNGQPENNYKTTPPVLDSDGSFFLYSRLTVDKSRWQEGNVFSCSVMHEALHNHYTQNSLSLSLGGGGGSGGGGSAPAPAPAPAPAPAPAPAPAPGGGGSGGGGSDHCPLGPGRCCRLHTVRASLEDLGWADWVLSPREVQVTMCIGACPSQFRAANMHAQIKTSLHRLKPDTVPAPCCVPASYNPMVLIQKTDTGVSLQTYDDLLAKDCHCI

SEQ ID NO: 118 - protein, 364 aa, synthetic construct
APEAAGGPSVFLFPPKPKDTLMISRTPEVTCVVVDVSQEDPEVQFNWYVDGVEVHNAKTKPREEQFNSTYRVVSVLTVLHQDWLNGKEYKCKVSNKGLPSSIEKTISKAKGQPREPQVYTLPPSQNEMTKNQVSLTCLVKGFYPSDIAVEWESNGQPENNYKTTPPVLDSDGSFFLYSRLTVDKSRWQEGNVFSCSVMHEALHNHYTQKSLSLSLGGGGGSGGGGSAPAPAPAPAPAPAPAPAPAPGGGGSGGGGSDHCPLGPGRCCRLHTVRASLEDLGWADWVLSPREVQVTMCIGACPSQFRAANMHAQIKTSLHRLKPDTVPAPCCVPASYNPMVLIQKTDTGVSLQTYDDLLAKDCHCI

SEQ ID NO: 119 - protein, 364 aa, synthetic construct
APEAAGGPSVFLFPPKPKDTLMISRTPEVTCVVVDVSQEDPEVQFNWYVDGVEVHNAKTKPREEQFNSTYRVVSVLTVLHQDWLNGKEYKCKVSNKGLPSSIEKTISKAKGQPREPQVYTLPPSQEEMTKNQVSLTCLVKGFYPSDIAVEWESNGQPENNYKTTPPVLDSDGSFFLYSRLTVDKSRWQEGNVFSCSVMHEALHNHYTQKSLSLSLGGGGGSGGGGSAPAPAPAPAPAPAPAPAPAPGGGGSGGGGSDHCPLGPGRCCRLHTVRASLEDLGWADWVLSPREVQVTMCIGACPSQFRAANMHAQIKTSLHRLKPDTVPAPCCVPASYNPMVLIQKTDTGVSLQTYDDLLAKDCHCI

SEQ ID NO: 120 - protein, 344 aa, synthetic construct
GGPSVFLFPPKPKDTLMISRTPEVTCVVVDVSQEDPEVQFNWYVDGVEVHNAKTKPREEQFNSTYRVVSVLTVLHQDWLNGKEYKCKVSNKGLPSSIEKTISKAKGQPREPQVYTLPPSQEEMTKNQVSLTCLVKGFYPSDIAVEWESNGQPENNYKTTPPVLDSDGSFFLYSRLTVDKSRWQEGNVFSCSVMHEALHNHYTQESLSLSLGGGGGSGGGGSGGGGSGGGGSGGGGSDHCPLGPGRCCRLHTVRASLEDLGWADWVLSPREVQVTMCIGACPSQFRAANMHAQIKTSLHRLKPDTVPAPCCVPASYNPMVLIQKTDTGVSLQTYDDLLAKDCHCI

SEQ ID NO: 121 - protein, 364 aa, synthetic construct
APEAAGGPSVFLFPPKPKDTLMISRTPEVTCVVVDVSQEDPEVQFNWYVDGVEVHNAKTKPREEQFNSTYRVVSVLTVLHQDWLNGKEYKCKVSNKGLPSSIEKTISKAKGQPREPQVYTLPPSQDEMTKNQVSLTCLVKGFYPSDIAVEWESNGQPENNYKTTPPVLDSDGSFFLYSRLTVDKSRWQEGNVFSCSVMHEALHNHYTQKSLSLSLGGGGGSGGGGSAPAPAPAPAPAPAPAPAPAPGGGGSGGGGSDHCPLGPGRCCRLHTVRASLEDLGWADWVLSPREVQVTMCIGACPSQFRAANMHAQIKTSLHRLKPDTVPAPCCVPASYNPMVLIQKTDTGVSLQTYDDLLAKDCHCI

SEQ ID NO: 122 - protein, 364 aa, synthetic construct
APEAAGGPSVFLFPPKPKDTLMISRTPEVTCVVVDVSQEDPEVQFNWYVDGVEVHNAKTKPREEQFNSTYRVVSVLTVLHQDWLNGKEYKCKVSNKGLPSSIEKTISKAKGQPREPQVYTLPPSQEEMTKNQVSLTCLVKGFYPSDIAVEWESNGQPENNYKTTPPVLDSDGSFFLYSRLTVDKSRWQEGNVFSCSVMHEALHNHYTQRSLSLSLGGGGGSGGGGSAPAPAPAPAPAPAPAPAPAPGGGGSGGGGSDHCPLGPGRCCRLHTVRASLEDLGWADWVLSPREVQVTMCIGACPSQFRAANMHAQIKTSLHRLKPDTVPAPCCVPASYNPMVLIQKTDTGVSLQTYDDLLAKDCHCI

SEQ ID NO: 123 - protein, 25 aa, synthetic construct
GGGGSGGGGSGGGGSGGGGSGGGGS

SEQ ID NO: 124 - protein, 40 aa, synthetic construct
GGGGSGGGGSGGGGSGGGGSGGGGSGGGGSGGGGSGGGGS

SEQ ID NO: 125 - protein, 28 aa, synthetic construct
GGGGAPAPAPAPAPAPAPAPAPAPGGGG

SEQ ID NO: 126 - protein, 40 aa, synthetic construct
GGGGSGGGGSAPAPAPAPAPAPAPAPAPAPGGGGSGGGGS

SEQ ID NO: 127 - protein, 40 aa, synthetic construct
GGGGSGGGGSEPEPEPEPEPEPEPEPEPEPGGGGSGGGGS